European Patent Application EP 4 310 178 A1, published January 24, 2024. Title: Method for producing cerebral organoid having aggregated tau protein. Applicant: Keio University. The sequence listing filed with the application follows.

SEQUENCE LISTING (2 sequences)

SEQ ID NO: 1 - protein, 441 aa, Homo sapiens
MAEPRQEFEVMEDHAGTYGLGDRKDQGGYTMHQDQEGDTDAGLKESPLQTPTEDGSEEPGSETSDAKSTPTAEDVTAPLVDEGAPGKQAAAQPHTEIPEGTTAEEAGIGDTPSLEDEAAGHVTQARMVSKSKDGTGSDDKKAKGADGKTKIATPRGAAPPGQKGQANATRIPAKTPPAPKTPPSSGEPPKSGDRSGYSSPGSPGTPGSRSRTPSLPTPPTREPKKVAVVRTPPKSPSSAKSRLQTAPVPMPDLKNVKSKIGSTENLKHQPGGGKVQIINKKLDLSNVQSKCGSKDNIKHVLGGGSVQIVYKPVDLSKVTSKCGSLGNIHHKPGGGQVEVKSEKLDFKDRVQSKIGSLDNITHVPGGGNKKIETHKLTFRENAKAKTDHGAEIVYKSPVVSGDTSPRHLSNVSSTGSIDMVDSPQLATLADEVSASLAKQGL

SEQ ID NO: 2 - protein, 441 aa, Homo sapiens
MAEPRQEFEVMEDHAGTYGLGDRKDQGGYTMHQDQEGDTDAGLKESPLQTPTEDGSEEPGSETSDAKSTPTAEDVTAPLVDEGAPGKQAAAQPHTEIPEGTTAEEAGIGDTPSLEDEAAGHVTQARMVSKSKDGTGSDDKKAKGADGKTKIATPRGAAPPGQKGQANATRIPAKTPPAPKTPPSSGEPPKSGDRSGYSSPGSPGTPGSRSRTPSLPTPPTREPKKVAVVRTPPKSPSSAKSRLQTAPVPMPDLKNVKSKIGSTENLKHQPGGGKVQIINKKLDLSNVQSKCGSKDNIKHVSGGGSVQIVYKPVDLSKVTSKCGSLGNIHHKPGGGQVEVKSEKLDFKDRVQSKIGSLDNITHVPGGGNKKIETHKLTFRENAKAKTDHGAEIVYKSPVVSGDTSPRHLSNVSSTGSIDMVDSPQLATLADEVSASLAKQGL